European Patent Specification EP 2 945 642 B1, published February 21, 2024. Title: FACTOR 1 PROTEIN, FACTOR 2 PROTEIN AND INHIBITORS THEREOF FOR USE IN TREATING OR PREVENTING DISEASES. Applicant: Medizinische Hochschule Hannover. The sequence listing filed with the application follows.

SEQUENCE LISTING (39 sequences)

SEQ ID NO: 1 - protein, 142 aa, Homo sapiens
VSEPTTVAFDVRPGGVVHSFSHNVGPGDKYTCMFTYASQGGTNEQWQMSLGTSEDHQHFTCTIWRPQGKSYLYFTQFKAEVRGAEIEYAMAYSKAAFERESDVPLKTEEFEVTKTAVAHRPGAFKAELSKLVIVAKASRTEL

SEQ ID NO: 2 - protein, 173 aa, Homo sapiens
MAAPSGGWNGVGASLWAALLLGAVALRPAEAVSEPTTVAFDVRPGGVVHSFSHNVGPGDKYTCMFTYASQGGTNEQWQMSLGTSEDHQHFTCTIWRPQGKSYLYFTQFKAEVRGAEIEYAMAYSKAAFERESDVPLKTEEFEVTKTAVAHRPGAFKAELSKLVIVAKASRTEL

SEQ ID NO: 3 - protein, 200 aa, Homo sapiens
SGCRAGTGARGAGAEGREGEACGTVGLLLEHSFEIDDSANFRKRGSLLWNQQDGTLSLSQRQLSEEERGRLRDVAALNGLYRVRIPRRPGALDGLEAGGYVSSFVPACSLVESHLSDQLTLHVDVAGNVVGVSVVTHPGGCRGHEVEDVDLELFNTSVQLQPPTTAPGPETAAFIERLEMEQAQKAKNPQEQKSFFAKYW

SEQ ID NO: 4 - protein, 254 aa, Homo sapiens
MAAASAGATRLLLLLLMAVAAPSRARGSGCRAGTGARGAGAEGREGEACGTVGLLLEHSFEIDDSANFRKRGSLLWNQQDGTLSLSQRQLSEEERGRLRDVAALNGLYRVRIPRRPGALDGLEAGGYVSSFVPACSLVESHLSDQLTLHVDVAGNVVGVSVVTHPGGCRGHEVEDVDLELFNTSVQLQPPTTAPGPETAAFIERLEMEQAQKAKNPQEQKSFFAKYWHIILGGAVLLTALRPAAPGPAPPPQEA

SEQ ID NO: 5 - protein, 262 aa, Homo sapiens
MAAASAGATRLLLLLLMAVAAPSRARGSGCRAGTGARGAGAEGREGEACGTVGLLLEHSFEIDDSANFRKRGSLLWNQQDGTLSLSQRQLSEEERGRLRDVAALNGLYRVRIPRRPGALDGLEAGGYVSSFVPACSLVESHLSDQLTLHVDVAGNVVGVSVVTHPGGCRGHEVEDVDLELFNTSVQLQPPTTAPGPETAAFIERLEMEQAQKAKNPQEQKSFFAKYWMYIIPVVLFLMMSGAPDTGGQGGGGGGGGGGGSGR

SEQ ID NO: 6 - DNA, 1067 bp, Homo sapiens
ggcggacgctccacgtgtccctcgccgcgccccgtctacccgcccctgccctgaggaccctagtccaacatggcggcgcccagcggagggtggaacggcgtcggcgcgagcttgtgggccgcgctgctcctaggggccgtggcgctgaggccggcggaggcggtgtccgagcccacgacggtggcgtttgacgtgcggcccggcggcgtcgtgcattccttctcccataacgtgggcccgggggacaaatatacgtgtatgttcacttacgcctctcaaggagggaccaatgagcaatggcagatgagtctggggaccagcgaagaccaccagcacttcacctgcaccatctggaggccccaggggaagtcctatctgtacttcacacagttcaaggcagaggtgcggggcgctgagattgagtacgccatggcctactctaaagccgcatttgaaagggaaagtgatgtccctctgaaaactgaggaatttgaagtgaccaaaacagcagtggctcacaggcccggggcattcaaagctgagctgtccaagctggtgattgtggccaaggcatcgcgcactgagctgtgaccagcagccctgttgcgggtggcaccttctcatctccggtgaagctgaaggggcctgtgtccctgaaagggccagcacatcactggttttctaggagggactcttaagttttctacctgggctgacgttgccttgtccggaggggcttgcagggtggctgaagccctggggcagagaacagagggtccagggccctcctggctcccaacagcttctcagttcccacttcctgctgagctcttctggactcaggatcgcagatccggggcacaaagagggtggggaacatgggggctatgctggggaaagcagccatgctccccccgacctccagccgagcatccttcatgagcctgcagaactgctttcctatgtttacccaggggacctcctttcagatgaactgggaagagatgaaatgttttttcatatttaaataaataagaacattaaaaagcaaaaaaaaaaaaaaaaaa

SEQ ID NO: 7 - DNA, 913 bp, Mus musculus
gagcgcctgcgcattgccccggaagcaagatggcagcccccagcggaggcttctggactgcggtggtcctggcggccgcagcgctgaaattggccgccgctgtgtccgagcccaccaccgtgccatttgacgtgaggcccggaggggtcgtgcattcgttctcccaggacgtaggacccgggaacaagtttacatgtacattcacctacgcttcccaaggagggaccaacgagcaatggcagatgagcctggggacaagtgaagacagccagcactttacctgtaccatctggaggccccaggggaaatcctacctctacttcacacagttcaaggctgagttgcgaggtgctgagatcgagtatgccatggcctactccaaagccgcatttgagagagagagtgatgtccccctgaaaagtgaggagtttgaagtgaccaagacagcagtgtctcacaggcctggggccttcaaagctgagctctccaagctggtgatcgtagccaaggcggcacgctcggagctgtgaccctcgcctgtcaagggccttcatgtccacgttcctcaggcacactgaccgggactacttgtctagggcactggttcccataggagctgccctgccctgcacaggtcacactgtgtcactccgcagaactctctgagcccggtcacctgttttgccagggaagatgcagggcatgtgcgggggtgggatggaaggacttcctggctttcctgaagtcaagatgtggtgtggtttcccctctgagccacagatgagtgtccccatcccaggaccactttctaaccccatccagggcagctccactcagaaggatgggaaaggatagaaaaaataaataaataagtagccaccttagtggtggctctgtggggtcaggactcaga

SEQ ID NO: 8 - DNA, 2048 bp, Homo sapiens
ttcctcccggcgtgctccgcggctcttggctcacagccgtcccttcgctggtgggaagaagccgagatggcggcagccagcgctggggcaacccggctgctcctgctcttgctgatggcggtagcagcgcccagtcgagcccggggcagcggctgccgggccgggactggtgcgcgaggggctggggcggaaggtcgagagggcgaggcctgtggcacggtggggctgctgctggagcactcatttgagatcgatgacagtgccaacttccggaagcggggctcactgctctggaaccagcaggatggtaccttgtccctgtcacagcggcagctcagcgaggaggagcggggccgactccgggatgtggcagccctgaatggcctgtaccgggtccggatcccaaggcgacccggggccctggatggcctggaagctggtggctatgtctcctcctttgtccctgcgtgctccctggtggagtcgcacctgtcggaccagctgaccctgcacgtggatgtggccggcaacgtggtgggcgtgtcggtggtgacgcaccccgggggctgccggggccatgaggtggaggacgtggacctggagctgttcaacacctcggtgcagctgcagccgcccaccacagccccaggccctgagacggcggccttcattgagcgcctggagatggaacaggcccagaaggccaagaacccccaggagcagaagtccttcttcgccaaatactggcacatcatcctggggggggccgtgttgctcacagccctgcgtcctgctgcgccagggcccgcgccaccgccacaggaggcctgatggatgtacatcattcccgtcgtcctgttcctcatgatgtcaggagcgccagacaccgggggccagggtgggggtgggggtgggggtggtggtgggggtagtggccggtgagggcccaggctggtcagcgtcccgtcttgcacacccaggggcctccctttctgctggagtcccctgtgtcctcagccatcccaagaagggtttgctggtccctcctttccccccgtcccacgaggccacctgggccagccccttgtcctctgccttctgctggcagaggagcagctggactggggcctttggcacagcagccggtgtctcctgcgcccgcctcccccatggccccatgcagccccaggggcttcccccctgcccatggagtagagcccgagatcctggccactatgccagttctgacctcgcatccccctaccccgagcccatgcagtctgggaacatgccgccttctctccagcctctgtgcctttgttccaggtggtctcaccctcctgtccctggctgggctaggtggtcctgtccaggctcctgcagcgcccccctcactttgacactggactaggatgcagcctcccttctgtgtccccttgagggtaccctgggtcccctcatcaggggcagaggcatgaaagagtcggggctggatggccgggggcttctgggcccgacgcctagtgcagcccctggggtcgtggtttgacatttgtctgcctggtgcaaacaaggaatccttgcctttaaggtgacaggccctccacaggcttccagacttgaaggaaaaggtttaagaaagaaaacaaaaccaacagttagtggagtcaaagcccagacactgtaaatagaaccccctccaccaccccccgccgcccagcatcctacctggactgcggtgctacgagggcctgcgggcctttgctgtgtgccaccctccctgtaagtctatttaaaaacatcgacgatacattgaaatgtgtgaacgttttgaaaagctacagcttccagcagccaaaagcaactgttgttttggcaagacggtcctgatgtacaagcttgattgaaattcactgctcacttgatacgttattcagaaacccaaggaatggctgtccccatcctcatgtggctgtgtggagctcagctgtgttgtgtggcagtttattaaactgtcccccagatcgacacgcaaaaaaaaaaaaaaa

SEQ ID NO: 9 - DNA, 1960 bp, Homo sapiens
ttcctcccggcgtgctccgcggctcttggctcacagccgtcccttcgctggtgggaagaagccgagatggcggcagccagcgctggggcaacccggctgctcctgctcttgctgatggcggtagcagcgcccagtcgagcccggggcagcggctgccgggccgggactggtgcgcgaggggctggggcggaaggtcgagagggcgaggcctgtggcacggtggggctgctgctggagcactcatttgagatcgatgacagtgccaacttccggaagcggggctcactgctctggaaccagcaggatggtaccttgtccctgtcacagcggcagctcagcgaggaggagcggggccgactccgggatgtggcagccctgaatggcctgtaccgggtccggatcccaaggcgacccggggccctggatggcctggaagctggtggctatgtctcctcctttgtccctgcgtgctccctggtggagtcgcacctgtcggaccagctgaccctgcacgtggatgtggccggcaacgtggtgggcgtgtcggtggtgacgcaccccgggggctgccggggccatgaggtggaggacgtggacctggagctgttcaacacctcggtgcagctgcagccgcccaccacagccccaggccctgagacggcggccttcattgagcgcctggagatggaacaggcccagaaggccaagaacccccaggagcagaagtccttcttcgccaaatactggatgtacatcattcccgtcgtcctgttcctcatgatgtcaggagcgccagacaccgggggccagggtgggggtgggggtgggggtggtggtgggggtagtggccggtgagggcccaggctggtcagcgtcccgtcttgcacacccaggggcctccctttctgctggagtcccctgtgtcctcagccatcccaagaagggtttgctggtccctcctttccccccgtcccacgaggccacctgggccagccccttgtcctctgccttctgctggcagaggagcagctggactggggcctttggcacagcagccggtgtctcctgcgcccgcctcccccatggccccatgcagccccaggggcttcccccctgcccatggagtagagcccgagatcctggccactatgccagttctgacctcgcatccccctaccccgagcccatgcagtctgggaacatgccgccttctctccagcctctgtgcctttgttccaggtggtctcaccctcctgtccctggctgggctaggtggtcctgtccaggctcctgcagcgcccccctcactttgacactggactaggatgcagcctcccttctgtgtccccttgagggtaccctgggtcccctcatcaggggcagaggcatgaaagagtcggggctggatggccgggggcttctgggcccgacgcctagtgcagcccctggggtcgtggtttgacatttgtctgcctggtgcaaacaaggaatccttgcctttaaggtgacaggccctccacaggcttccagacttgaaggaaaaggtttaagaaagaaaacaaaaccaacagttagtggagtcaaagcccagacactgtaaatagaaccccctccaccaccccccgccgcccagcatcctacctggactgcggtgctacgagggcctgcgggcctttgctgtgtgccaccctccctgtaagtctatttaaaaacatcgacgatacattgaaatgtgtgaacgttttgaaaagctacagcttccagcagccaaaagcaactgttgttttggcaagacggtcctgatgtacaagcttgattgaaattcactgctcacttgatacgttattcagaaacccaaggaatggctgtccccatcctcatgtggctgtgtggagctcagctgtgttgtgtggcagtttattaaactgtcccccagatcgacacgcaaaaaaaaaaaaaa

SEQ ID NO: 10 - DNA, 1627 bp, Mus musculus
gggctgtatggctctcggtttttctcaacgctcccgtatggtggccgcgggtgccggggtgacccggctgctagtgctcttgctgatggtagccgcggctcctagcagagcccgaggcagcggctgccgggtcggggcctccgcgcgtgggaccggggccgatggccgtgaagctgagggctgtggcaccgtggctttgctgctggagcattcatttgagctcggtgatggagccaacttccagaagcgaggcttgctgctctggaaccagcaggatggcaccctgtcggcaacacagcgacagctcagtgaggaggagcgtggccgactccgggatgtggctgctgtcaatggcctctacagggtccgggtcccgaggcggcctgggacacttgatggttcagaagctggcggccatgtgtcttccttcgtcccagcgtgctccctggtggagtcgcacctttcggaccagctgaccttgcacgtggatgtggctggcaacgtggtgggcctgtctgtggtggtgtaccctgggggctgccggggctccgaggtggaagatgaggacctggagctgttcaatacatctgtgcagctgcggcctcccagcactgctccaggccccgagactgcagccttcattgagcgcctggagatggagcaggcccagaaggccaagaacccacaggagcagaagtctttctttgccaaatactggcacctcatcctggggggggccgtgttgctcacagccctacgtcctgctgccccagggcctgcaccagcgccaacggaggcctaatggatgtacatcattccagttgtgctgttcctcatgatgtcgggagcgccggacgctgggggccagggcggcggtgggggcgggggcagcagccggtgagcagctgtgccacctagagccccccccagagccagcccaagaaggagttcctgtccccacatttccctattgcatgaatatggaaggctgtcccttcagtgagccctctggccttcctgtaagcccctctttctgtccctgagcctctctctcatcctgttgactgagagcttgggtggacctccctgtagccagctcactgcaactgtgtcccaccatgtggcactgtgctcctctgtctgctaaacacccaccagcctgccccaccccaccccaccatacactttgggaacttgccaagctctctccagcctctgtgcctttgccctgcaggccccgtgcgcccctcactgtcactctccagccctttgccaaggatctgtggcccagaggcctctgctcttagtggctaggtcagcctccagcccactgtccaggtggcatgctgtcttctttgcccccctctctggtgccccagaataccatggtgacctaccactatcctttctgcctttggatgtcatagcctggatctgtcaccaggagaggattgtgggcctccacgttagtctgtgaatgcacacttcgagtgacttgtgtgcaggttttgagagccggttttgcactagctgctcgacagctgctggcatggccgtgctcttgcacatgcgccgctgtgggcatggggattgctgtgcagcctcagctgtgttgtgtggctgctga

SEQ ID NO: 11 - DNA, 1855 bp, Mus musculus
gagaaatggccgccctgactgcgggagcaggcggacgggcgctagtgcgcaggcgcggcgtgcggcgcaggcgcgtgagcctcaggatgaaccctgtgtttcctagcgggctgtatggctctcggtttttctcaacgctcccgtatggtggccgcgggtgccggggtgacccggctgctagtgctcttgctgatggtagccgcggctcctagcagagcccgaggcagcggctgccgggtcggggcctccgcgcgtgggaccggggccgatggccgtgaagctgagggctgtggcaccgtggctttgctgctggagcattcatttgagctcggtgatggagccaacttccagaagcgaggcttgctgctctggaaccagcaggatggcaccctgtcggcaacacagcgacagctcagtgaggaggagcgtggccgactccgggatgtggctgctgtcaatggcctctacagggtccgggtcccgaggcggcctgggacacttgatggttcagaagctggcggccatgtgtcttccttcgtcccagcgtgctccctggtggagtcgcacctttcggaccagctgaccttgcacgtggatgtggctggcaacgtggtgggcctgtctgtggtggtgtaccctgggggctgccggggctccgaggtggaagatgaggacctggagctgttcaatacatctgtgcagctgcggcctcccagcactgctccaggccccgagactgcagccttcattgagcgcctggagatggagcaggcccagaaggccaagaacccacaggagcagaagtctttctttgccaaatactggatgtacatcattccagttgtgctgttcctcatgatgtcgggagcgccggacgctgggggccagggcggcggtgggggcgggggcagcagccggtgagcagctgtgccacctagagccccccccagagccagcccaagaaggagttcctgtccccacatttccctattgcatgaatatggaaggctgtcccttcagtgagccctctggccttcctgtaagcccctctttctgtccctgagcctctctctcatcctgttgactgagagcttgggtggacctccctgtagccagctcactgcaactgtgtcccaccatgtggcactgtgctcctctgtctgctaaacacccaccagcctgccccaccccaccccaccatacactttgggaacttgccaagctctctccagcctctgtgcctttgccctgcaggccccgtgcgcccctcactgtcactctccagccctttgccaaggatctgtggcccagaggcctctgctcttagtggctaggtcagcctccagcccactgtccaggtggcatgctgtcttctttgcccccctctctggtgccccagaataccatggtgacctaccactatcctttctgcctttggatgtcatagcctggatctgtcaccaggagaggattgtgggcctccacgttagtctgtgaatgcacacttcgagtgacttgtgtgcaggttttgagagccggttttgcactagctgctcgacagctgctggcatggccgtgctcttgcacatgcgccgctgtgggcatggggattgctgtgcagcctcagctgtgttgtgtggctgctgattaaactgtcccctaaacagccactcttcagctcacttcctgccttctgtgcttgtgaatagtcctgagttgccgctgtggtttgcctggtttatgtttgaatggctttcttagggtatgttacagaggggtgcctgagcagattaaagttgctgtgagcaaggacgccttccgaactctgggaggaggctggttcctgaccctccta

SEQ ID NO: 12 - protein, 173 aa, Macaca mulatta
MAAPSGGWNGVGASLWAALLLGAVALSPAEAVSEPTTVAFDVRPGGVVHSFSHNVGPGDKYTCMFTYASQGGTNEQWQMSLGTSEDHQHFTCTIWRPQGKSYLYFTQFKAEVRGAEIEYAMAYSKAAFERESDVPLKTEEFEVTKTAVAHRPGAFKAELSKLVIVAKASRTEL

SEQ ID NO: 13 - protein, 166 aa, Mus musculus
MAAPSGGFWTAVVLAAAALKLAAAVSEPTTVPFDVRPGGVVHSFSQDVGPGNKFTCTFTYASQGGTNEQWQMSLGTSEDSQHFTCTIWRPQGKSYLYFTQFKAELRGAEIEYAMAYSKAAFERESDVPLKSEEFEVTKTAVSHRPGAFKAELSKLVIVAKAARSEL

SEQ ID NO: 14 - protein, 174 aa, Bos taurus
MAAPSGRRNGSGGANLWVSLLLAAAALRPVETVSEPTTVAFDVRPGGVVHSFSQNVGPGDKYTCVFTYASQGGTNEKWQMSLGTSEDHQHFTCTIWRPQGKSYLYFTQFKAEVRGAEIEYGMAYSKAAFEKESDVPLKNEEFEVTKTAVFHRPGAFKAELSKLVIVAKATRSEL

SEQ ID NO: 15 - protein, 174 aa, Loxodonta africana
MAAPRGRRNGSAGASMWGALLLAAVALRSVEAVSEPTTVAFDVRPGGVVHSFSHSAGPGDRFTCTFTYASQGGTNEQWQMSLGTSEDHQHFTCTIWRPQGKSYLYFTQFKAEVRGAQIEYGMAYSKAASERESDVPLKNEEFEVTKTTVAHRPGAFKAELSKLVIVAKASHSEL

SEQ ID NO: 16 - protein, 173 aa, Heterocephalus glaber
MAAPRGNSDGCGGAWFAALLLAAVALRPAEAVSEPTTVAFDVRPGGVVHSFSQNVGPGDKFTCTFTYASQGGTNEQWQMSLGTSEDHQHFTCIIWRPQGKSYLYFTQFKAEVHGAEIEYAMAYSKAAFERESDVPLKNEEFEVTKAAVAHRPGAFRAELSKLVIVAKEAHSEL

SEQ ID NO: 17 - protein, 173 aa, Mustela putorius furo
MAAPSERRNGGGASLWAALLLAAAALRPAEAVSEPTTVAFDVRPGGVVHSFSQNVGPGDKYTCAFTYASQGGTNEKWQMSLGISEDHQHFTCTIWRPQGKSYLYFTQFRAEVRGAEIEYGMAYSKAAFERESDVPLKSEEFEVTKTAVSHRPGAFKAELSKLVIVAKASRSEL

SEQ ID NO: 18 - protein, 167 aa, Gallus gallus
MAAPCGRSSRWLWAAVVPAAVLCLAVRAAEEASTAEFDVRPGGEVHFFSRSLGDYTCTFTYSAQGGTNEQWQMNIGVSEDNLLFSCSVWRPQGKSYLFFTQFKAEVKGAKIEYAMAYSQAAVGAQSDIPLKQEEFEITETTVSHREGKFRFELSKLMIVAKTPHDEL

SEQ ID NO: 19 - protein, 169 aa, Oreochromis niloticus
MARQSNTCAGNLAFLFALALIAARVPAEASEEQAKTVEFNVKPGGVVHTFSEGIGEYECSFTYASQGGTNEQWLMSVGLTDDNRLFSCSVWRPQGKSYLFFTQFKAELKGTKIEYANAYSQSAAGGQSDVPLKPEEFTIGESTVTHKDGKFSAQLSKLTVIGRTQKDEL

SEQ ID NO: 20 - protein, 158 aa, Xenopus tropicalis
MATYGIICAFLLLLAVCSAQEKSSTEEFDVRPGGLQHSFTSKLGDYACTFTYAAQGGTNEKWHMSVGLSDDNQHFSCSIWRPQGKSYLFFTGFKAEVTGGKIEFSEAYSQASSDGSSDVKLKSSEYDVTDNVVSHRPGSFSSSLCKLVLVARSEHDEL

SEQ ID NO: 21 - protein, 254 aa, Macaca mulatta
MAATSGGATRLLLLLLMAVAAPSRARGSGCRAGTGARGAGAEGREGEACGTVGLLLEHSFEIDDSANFRKRGSLLWNQQDGTLSLSQRQLSEEERGRLRDVAALNGLYRVRVPRRPGALDGLEASGYVSSFVPACSLVESHLSDQLTLHVDVAGNVVGVSVVTHPGGCRGHEVEDVDLELFNTSVQLQPPATAPGPETAAFIERLEMEQAQKAKNPQEQKSFFAKYWHIILGGAVLLTALRPAAPGPAPPPQEA

SEQ ID NO: 22 - protein, 254 aa, Cavia porcellus
MAAAGAGAPRLLLLLLIVAAAPSRARGSSCRAGAATRGVGAEGREGESCGTVGLLLEHSFEIDDTAQFRKRGSLLWNQQDGTLSLSQRQLNEEERGRLRDVAALNGLYRVRVPRRPGALDSAEAGGYVSSFVPACSLVESHLSDQLTLHVDVAGNVVGVSVVTYPGGCRGHEVEDVDLELFNTSVRLRPPGTAPGPETAAFIERLEMEQAQKAKNPQEQKSFFAKYWHLILGGAVLLTALRPAAPGPTPPPQEA

SEQ ID NO: 23 - protein, 254 aa, Canis lupus familiaris
MAAAGAVVTRLFLLLLMAAAAPSRARGSGCRSGAALRGAGAEGRESEGCGTVGLLLEHSFEIDDSAHFRKRGSLLWNQQDGTLSLSQRQLNEEERGRLRDVAALNGLYRVRVPQRPGVPDGAEAGGYVSSFVPACSLVESHLSDQLTLHVDVAGNVVGVSVVTHPGGCRGHEVEDVDLELFNTSVHLQPPATAPGPETAAFIERLEMEQAQKAKNPQEQKSFFAKYWHLVLGGAVLLTALRPAAPGPTPPPQEA

SEQ ID NO: 24 - protein, 254 aa, Mus musculus
MVAAGAGVTRLLVLLLMVAAAPSRARGSGCRVGASARGTGADGREAEGCGTVALLLEHSFELGDGANFQKRGLLLWNQQDGTLSATQRQLSEEERGRLRDVAAVNGLYRVRVPRRPGTLDGSEAGGHVSSFVPACSLVESHLSDQLTLHVDVAGNVVGLSVVVYPGGCRGSEVEDEDLELFNTSVQLRPPSTAPGPETAAFIERLEMEQAQKAKNPQEQKSFFAKYWHLILGGAVLLTALRPAAPGPAPAPTEA

SEQ ID NO: 25 - protein, 254 aa, Equus caballus
MAAAGAGATRLLLLLLMAAAAPSRARGSGCRPGTAARGAGAEGREGEGCGPVGLLLEHSFEIDDNAHFRKRGSLLWNQQDGTLSLSQRQLSEEERGRLRDVAALNGLYRVRVPRRPGTPDGLEAGGYVSSFVPACSLVESHLSDQLTLHVDVAGNVVGVSVVTHPGGCRGHEVEDVDLELFNTSVQLQPPVTAPGPETAAFIERLEMEQAQKAKNPQEQKSFFAKYWHLILGGAVLLTALRPAAPGPAPPPQEA

SEQ ID NO: 26 - protein, 258 aa, Xenopus laevis
GGQRAGPLSSIVTGNCWVWLIALPFLAVTAQGSVCRLKTGDGRESESCGTNLELEHSFELDDSIHFTKRGSLFWSGTAEQSISILQKQLTEDERNKLRDIANLNGLYRIRIPRKLGITEEANEYVTSFVRACSMVESHLSDEITVHTDLSGNVIGVSIVTFPGSCNGAEVEDVDLEMFNTTVHMQQPIPAAVPETAAFIERLEMEQAQKAKNPQEQKSFFAKYWMYIIPVVLFLMMSGASDAGNQGGNGGGGGGGGGR

SEQ ID NO: 27 - protein, 251 aa, Danio rerio
MAPIRVLSLVLPILSTVPLLLTQFGECNNGRRSGDAVDTDFSGFSVPLEHSFEVDDVPRFRLRGALQFRGGRENSVYLSQNQLSEKDRNTLKDVAAVDGLYRIRVPRVSLQVDRQTERQYEGYLTAFVRACALVESHLSDVITLHTDVSGYVIGISIVTIPGSCRGIEVEDEVDLEVFNTTISVMAPVTAPVPETAPYIERMEMEMEKKGKNPQEQKSFFAKYWYLILGGAVFLMATSSAQTPPGGAREQS

SEQ ID NO: 28 - protein, 262 aa, Pan troglodytes
MAAASAGATRLLLLLLMAVAAPSRARGSSCRAGTGARGAGAEGREGEACGTVGLLLEHSFEIDDSANFRKRGSLLWNQQDGTLSLSQRQLSEEERGRLRDVAALNGLYRVRIPRRPGALDGLEAGGYVSSFVPACSLVESHLSDQLTLHVDVAGNVVGVSVVTQPGGCRGHEVEDVDLELFTTSVQLQPPTTAPGPETAAFIERLEMEQAQKAKNPQEQKSFFAKYWMYIIPVVLFLMMSGAPDTGGQGGGGGGGGGGGSGR

SEQ ID NO: 29 - protein, 258 aa, Mus musculus
MVAAGAGVTRLLVLLLMVAAAPSRARGSGCRVGASARGTGADGREAEGCGTVALLLEHSFELGDGANFQKRGSLLWNQQDGTLSATQRQLSEEERGRLRDVAAVNGLYRVRVPRRPGTLDGSEAGGHVSSFVPACSLVESHLSDQLTLHVDVAGNVVGLSVVVYPGGCRGSEVEDEDLELFNTSVQLRPPSTAPGPETAAFIERLEMEQAQKAKNPQEQKSFFAKYWMYIIPVVLFLMMSGAPDAGGQGGGGGGGSSR

SEQ ID NO: 30 - protein, 210 aa, Heterocephalus glaber
MVMAASGASASRLLLLLLIVAAAPSRARGSGCRAGAAARGVGAEGREGESCGTVGLLLEHSFEIDDAAHFRKRGSLLWNQQDGTLSPSQRQLSEEERGRLRDVAALNGLYRVRVPRRPGALDSSEAGGYVSSFVPACSLVESHLSDQLTLHVDVAGNVVGVSVVTDPGGCRGHEVEDVDLELFNTSVQLQPPGTAPGPETAAFIERLEME

SEQ ID NO: 31 - protein, 262 aa, Loxodonta africana
MAAAGAGATRLLLLLLMAAAAPSRARGSSCRAGAATRGAGAEGRENEGCGTVGLLLEHSFEIDDAMHFRKRGSLLWNQQDGTLSLSQRQLSEEERGRLRDVAALNGLYRVRVPRRPGAPEGPEAGGYVSSFVPACSLVESHLSDQLTLHVDVVGNVVGVSVVTLPGGCRGYEVEDVDLELFNTTVQLQPPTTAPGPETAAFIERLEMEQAQKAKNPQEQKSFFAKYWMYIIPVVLFLMMSGAPDTGGQGGGGGGGGGGGSGR

SEQ ID NO: 32 - protein, 263 aa, Xenopus tropicalis
MAAGCLVGQRAGPLSDKLSGYCWVLLPLLLVATAQASVCRLKTGDGRDSESCGTNLELEHSFELDDSIHFKKRGSLIWSGTAEQSISILQKQLTEDERNKLRDIANLNGLYRIRVPRKLGITEEANEYVTSFVRACSMVESHLSDQISVHTDISGNVVGISIVTFPGSCNGAEVEDVDLEMFNTTVYIQQPIAAAVPETAAFIERLEMEQAQKAKNPQEQKSFFAKYWMYIIPVVLFLMMSGASDAGNQGGNGGGGGGSGGGR

SEQ ID NO: 33 - protein, 251 aa, Danio rerio; identical to SEQ ID NO: 27

SEQ ID NO: 34 - protein, 269 aa, Homo sapiens [sequence omitted]

SEQ ID NO: 35 - protein, 31 aa, Homo sapiens
MAAPSGGWNGVGASLWAALLLGAVALRPAEA

SEQ ID NO: 36 - protein, 6 aa, Artificial Sequence
  Hexahistidin-tag for purification of proteins
HHHHHH

SEQ ID NO: 37 - protein, 27 aa, Homo sapiens
MAAASAGATRLLLLLLMAVAAPSRARG

SEQ ID NO: 38 - protein, 16 aa, Homo sapiens
CTIWRPQGKSYLYFTQ

SEQ ID NO: 39 - protein, 16 aa, Homo sapiens
CEQAQKAKNPQEQKSF